European Patent Application EP 4 324 930 A2, published February 21, 2024. Title: COMPOSITIONS AND METHODS FOR PERONOSPORA RESISTANCE IN SPINACH. Applicant: Seminis Vegetable Seeds, Inc. Application EP. The sequence listing filed with the application follows.

SEQUENCE LISTING (25 sequences)

SEQ ID NO: 1 - DNA, 93 bp, Spinacia oleracea
  source 1..93: mol_type = genomic DNA
taggggtaattaaccaaattggtattaaattatacccatttgccctgttggtgtaaaggtcgatggatgagtataaatattactctctccgtc

SEQ ID NO: 2 - DNA, 70 bp, Spinacia oleracea
  source 1..70: mol_type = genomic DNA
tggggctaattaaccagattggtattaacttatacccatttgccacgttggtgtaaaggtcgatggatgg

SEQ ID NO: 3 - DNA, 93 bp, Spinacia oleracea
  source 1..93: mol_type = genomic DNA
taggggtaattaaccagattggtattaaattatacccatttgccacgttggtgtaaaggtcgatggatgagtataaatattactctctctgtc

SEQ ID NO: 4 - DNA, 102 bp, Spinacia oleracea
  source 1..102: mol_type = genomic DNA
aaggtttgatgctgcaagagaaaagtagatttagaaacgggtaaacagtgaaaaaaagatggaatattactcatactataacatttgtttcaaggaaaccat

SEQ ID NO: 5 - DNA, 100 bp, Spinacia oleracea
  source 1..100: mol_type = genomic DNA
aaggtttgacgctgcaagacaaaggtagatttagaaacgggtcaacagtaaaaaaaagatggaattactcatactataacatttgtttcaaggaaaccat

SEQ ID NO: 6 - DNA, 100 bp, Spinacia oleracea; identical to SEQ ID NO: 5
  source 1..100: mol_type = genomic DNA

SEQ ID NO: 7 - DNA, 101 bp, Spinacia oleracea
  source 1..101: mol_type = genomic DNA
aagttatgttaggcttgggaatggaaggttattcactgggacgtctatttataaagggagggtgaatttgtccgtcaagaagttgtacccgattgtgtata

SEQ ID NO: 8 - DNA, 101 bp, Spinacia oleracea
  source 1..101: mol_type = genomic DNA
aagttatgttaggcttgggaatggaaggttattcactgggacgtctatttataaagggaggatgaatttgtccgtcaagaagttgtacccgattgtgtata

SEQ ID NO: 9 - DNA, 100 bp, Spinacia oleracea
  source 1..100: mol_type = genomic DNA
taatatcaatattttttatataaaccattttaataaattattcccttcgtcccttaatattcgacccgatttgactttttgcactgttacataattcaat

SEQ ID NO: 10 - DNA, 101 bp, Spinacia oleracea
  source 1..101: mol_type = genomic DNA
taatatcaatattttttataaaaaccattttaataaattactccctccgtctcttaatactcgactcgctttgactttttgcactatttacataattcaat

SEQ ID NO: 11 - DNA, 101 bp, Spinacia oleracea; identical to SEQ ID NO: 10
  source 1..101: mol_type = genomic DNA

SEQ ID NO: 12 - DNA, 103 bp, Spinacia oleracea
  source 1..103: mol_type = genomic DNA
ttgaatgagaactttgattttagaaaggaagataacaacaagttttctgtttttcacaaaattaaaaaatcaaaatataaaaatcacaaaaagtaattttcag

SEQ ID NO: 13 - DNA, 104 bp, Spinacia oleracea
  source 1..104: mol_type = genomic DNA
ttgaatgagaactttgattttagaaaggaagacaacaacaagttttctgttttttacaaaattaaaaaatcaaaatataaaaatcacgaaaagtaatttttcag

SEQ ID NO: 14 - DNA, 100 bp, Spinacia oleracea
  source 1..100: mol_type = genomic DNA
ttgaatgagaactttgattttagaaaggaagacaacaacaagttttctgtttttcacaaaattaaaaatcaaaatataaaaatcacgaaaagtaattttc

SEQ ID NO: 15 - DNA, 101 bp, Spinacia oleracea
  source 1..101: mol_type = genomic DNA
aactaacactactaaaaaatgatgtgattttttattttattttttcatctaaaaaaagaaaagaacaagaaacccccaatcacaccgtaacccttaaaaag

SEQ ID NO: 16 - DNA, 101 bp, Spinacia oleracea
  source 1..101: mol_type = genomic DNA
aactaacactactaaaaaatgatgtgattttttattttattttttcatctaagaaaagaaaagaacaagaaacccccaatcacaccgtaacccttaaaaag

SEQ ID NO: 17 - DNA, 101 bp, Spinacia oleracea; identical to SEQ ID NO: 16
  source 1..101: mol_type = genomic DNA

SEQ ID NO: 18 - DNA, 101 bp, Spinacia oleracea
  source 1..101: mol_type = genomic DNA
ggctcaatgtcatgttttctacaaaatggcacccataactcggcaaagctagctgcctcagccattgcctcgaaagttaggagagcgccgccatcatcgga

SEQ ID NO: 19 - DNA, 101 bp, Spinacia oleracea; identical to SEQ ID NO: 18
  source 1..101: mol_type = genomic DNA

SEQ ID NO: 20 - DNA, 101 bp, Spinacia oleracea
  source 1..101: mol_type = genomic DNA
ggctcaatgtcatgttttctacaaaatggcacccataactcggcaaagctagctgcttcagccattgcctcgaaagttaggagagcgccgccatcatcgga

SEQ ID NO: 21 - DNA, 102 bp, Spinacia oleracea
  source 1..102: mol_type = genomic DNA
gcaatcgttacatattgtaaatctgcatataataaaaattataaaaaaataaattgatattctaaaacattttaattgtcgcaacttacgaacctttatcat

SEQ ID NO: 22 - DNA, 102 bp, Spinacia oleracea
  source 1..102: mol_type = genomic DNA
gcaatcgttacatattgtaaatctgcatataataaaaattgtaaaaaaataaattgatattctaaaacattttaattgtcgcaacttacgaacctttatcat

SEQ ID NO: 23 - DNA, 102 bp, Spinacia oleracea
  source 1..102: mol_type = genomic DNA
gcaatcgttacatattgtaaatctgcatataataaaaattataaaaaaataaattgatattctaaaacattttaattgtggcaacttacgaacctttatcat

SEQ ID NO: 24 - DNA, 239 bp, Spinacia oleracea
  source 1..239: mol_type = genomic DNA
aaaatgcaacacaatctatcttaacctaatcattaagttgaataatcaactattaacccaaaaaatgactgctcttatcattaagttgaataatcagtagatattgcctagtgaaccatcaaacaaattaaaaatgcaacacaatctatcttaacctaatcattaagttgaataatcaactattaacccgaaaaatggctgctcttttaaacctttgaaacccgttcatctttctcaac

SEQ ID NO: 25 - DNA, 198 bp, Spinacia oleracea
  source 1..198: mol_type = genomic DNA
agaatcgtcctgttaatcgatctaaaccctcttctccacctccaaaaccctaaatcttacatcacttcaatcctcacttccgccaaaattctcctctcatttccccctctttctctttccctatcctccttcaagctcttcttctcttctctatctcctctcaaatcgtcatcctcgctccccaacttcccaatttca